European Patent Specification EP 4 098 658 B1, published September 4, 2024. Title: Novel protein variant and a method for producing L-lysine using the same. Applicant: CJ CheilJedang Corporation. The sequence listing filed with the application follows.

SEQUENCE LISTING (10 sequences)

SEQ ID NO: 1 - protein, 985 aa, Artificial Sequence
  (D676Y)_NCgl0752_amino acid
MSTGLTPPPQPIKRPPKAVTWIFAIIALVILIAPMSVGFYTDWLWFGEVDFRGVFSKVIVTRIVLFVIFALIAGFVTWLAGYFVTKLRPDEMSAFDTQSPVYQYRQMIENSLRRVMVIIPIFVALLAGLIGQRSWRTVQMWLNGQDFGVSDQQFGLDYGFYAFDLPMLRLIADSLSMMLIVAFLIALVGHYLMGGIRAGNQMTGQKSFVSRGARTQLAVTAGLWMLVKVAGYWLDRYDLLTKENSTFTGASYTDINAQLPAKIILLVIALFVAIAFFSAIFLKDLRIPGLAVVLMLLSSVIIGAAWPLMLERFSVQPNRAEKEAEYISRNIESTRYAYGITDEDVTYEENWGAGETTNEEVAADSATISNIRLLDPQILSPTFTQQQQLRNFYGFPDQLAMDRFEVDGKLRDFVVAARELDPNALQQNQQDWINRHTVYTHGNGFIAAQANQVDEVARDVGSTRGGYPVYTVSDLQSNARAAESEDAEELGIKVDEPRVYYGPLIASATDGADYAIVGDTGDGPVEYDTDTSSYTYEGAGGVDIGNMVNRAMFALRYQEMNMLLSDRVGSESKILFERDPRSRVEKVAPWLTTDSKTYPTVIDGRIKWIVDGYTTLDSLPYSTRTSLTEATQDAVMPDGTPQPLITDRVGYIRNSVKAVVDAYDGTVELYEFDTEYPVLKAWRGVFPDTVKDGSEISDELRAHLRYPEDLFKVQRDMLAKYNVDDSGTFFTNDAFWSVPGDPTAAEGRQELKQPPYYVVAADPETGESSFQLITPFRGLQREYLSAHMSASSDPVTYGEITVRVLPTDSVTQGPKQAQDAMMSSDQVAQDQTLWRGSNDLHNGNLLTLPVGGGEILYVEPIYSQRKDQASAFPKLLRVLVFYKGQVGYAPTIAEALSQVGIDPKEAQDIEEVDGTATTPSTDETDTDTDQPATETPTAPVSEAEGIAAINDALSNLEAARDSSFEEYGRALDALDRAVDSYQSAQ

SEQ ID NO: 2 - DNA, 2958 bp, Artificial Sequence
  (D676Y)_NCgl0752_nucleic acid
ttgtcgactggtctcacacctcctccccaaccgatcaagcgacctcccaaggcggtgacatggatcttcgccattatcgcgttggtcattctcatcgccccaatgagtgttggcttctataccgactggctttggttcggtgaagtcgatttccgaggcgttttcagcaaggttattgtcactcgcattgttctctttgtgatctttgcgctaattgctgggtttgtcacatggcttgctggttattttgtgacaaaacttcgacctgatgagatgtcggcgtttgatacccagtcgcctgtgtatcagtaccgtcagatgatcgaaaacagccttcgtcgcgttatggtgatcattccaattttcgtcgcgttgctggctggcctaattggtcagcgttcgtggcgcaccgttcaaatgtggctgaatggccaggactttggcgtttcggatcagcagttcggcttggattatggattctacgcgtttgatcttccgatgcttcgcctcatcgctgactcactgtcgatgatgttgatcgttgctttcctgatcgcactcgttggccattacctcatgggtggcattcgcgctggaaaccagatgacgggccagaagtcctttgtatcccgtggtgcgcgcactcagcttgcggtaactgctggtctgtggatgcttgttaaggtcgctggctactggctggatcgctatgacctgctgactaaggaaaactcaaccttcacaggtgcaagctacaccgacatcaatgcacagctgccagcgaagatcatcctgctggttatcgcattgttcgtggcgatcgcgttcttctctgcgatcttcctgaaggacctccgcatcccaggtcttgccgtagttctgatgctgctgagctctgtgatcattggtgctgcttggcctttgatgctggagcgtttctccgttcagccaaaccgtgcagaaaaagaagccgagtacatttctcgaaacattgaatcgactcgctatgcctatggcatcaccgatgaagatgtcacctacgaggaaaactggggagcaggggagaccaccaatgaagaagtcgccgctgattctgcaacgatttctaacattcgtctgctggatccacagatcctgtcaccaaccttcacccagcaacagcagctgcgaaacttctacggtttcccagaccagctggcgatggaccgctttgaagtagatggcaaactccgcgactttgttgtggcagcacgtgagctcgatccaaacgccctgcagcaaaaccagcaggactggattaaccgtcacactgtttatacccacggcaacggcttcattgcagctcaagcaaaccaggtggatgaggtcgcccgcgacgtcggatccactcgtggtggttaccctgtctacaccgtctctgatttgcagtcgaatgctcgtgctgcagaaagcgaagatgctgaggagcttggcatcaaggttgatgagcctcgtgtgtactacggaccactgattgcttctgcgactgatggtgctgactacgcaattgtcggtgacaccggcgatggcccagtcgagtacgacactgacacctccagctacacctacgaaggtgctggcggcgtggacattggaaacatggtcaaccgtgcgatgtttgcattgcgctaccaggaaatgaacatgctcctgtctgatcgtgttggttccgaatccaagatcctatttgagcgcgatcctcgttcccgtgtggaaaaggttgcaccttggttgaccactgactccaagacctacccaactgtgattgatggtcgcatcaagtggatcgtcgatggctacaccaccttggatagtcttccgtactccacgcgcacctcactgacggaagcgactcaggatgctgtcatgcctgacggcaccccacagccactgatcacagatagggtcggttacatccgcaactccgtgaaggctgttgttgatgcgtacgacggaactgttgaactctacgaattcgacaccgaatatcctgttctgaaggcatggcgtggcgtgttcccagacaccgtgaaggacgggtcggagatttccgatgagcttcgcgcacacctgcgttacccagaagatttgttcaaggtccagcgtgacatgctggccaagtacaacgttgatgattctggaacattcttcaccaacgatgcgttctggtctgtcccaggtgacccaactgcagcggagggccgccaggaacttaagcagcctccttactacgtggtggcagcagacccagagaccggtgagtccagcttccagctgatcaccccgttccgtggacttcagcgcgagtacctctctgcacacatgtctgcgtcgtctgatccagttacctacggtgaaatcactgttcgtgtgctgcctaccgattctgtgacccagggtccaaagcaggcccaggatgcgatgatgtcatctgaccaggttgctcaggaccaaacactgtggcgtggatcgaacgatctgcacaacggaaacctgttgaccttgccagttggtggcggagagatcctctacgttgagccgatttactcgcagcgcaaggatcaggcatcggccttcccgaagcttctgcgcgtgctggtcttctacaagggtcaggttggttacgcaccaacgatcgctgaagccctatcgcaggtcggcattgatccgaaggaagcgcaggacatcgaagaggtagatggcaccgctacgacgccatcgactgatgagactgacactgacactgatcagcctgcaaccgaaaccccaactgcaccagtgagtgaggcggaaggaatcgcggccatcaacgatgcgttgagcaaccttgaagctgctcgcgatagctctttcgaagagtatggtcgtgcactcgatgcgcttgatcgtgccgtcgatagctaccagtccgcacagtag

SEQ ID NO: 3 - protein, 985 aa, Artificial Sequence
  (WT)_NCgl0752_amino acid
MSTGLTPPPQPIKRPPKAVTWIFAIIALVILIAPMSVGFYTDWLWFGEVDFRGVFSKVIVTRIVLFVIFALIAGFVTWLAGYFVTKLRPDEMSAFDTQSPVYQYRQMIENSLRRVMVIIPIFVALLAGLIGQRSWRTVQMWLNGQDFGVSDQQFGLDYGFYAFDLPMLRLIADSLSMMLIVAFLIALVGHYLMGGIRAGNQMTGQKSFVSRGARTQLAVTAGLWMLVKVAGYWLDRYDLLTKENSTFTGASYTDINAQLPAKIILLVIALFVAIAFFSAIFLKDLRIPGLAVVLMLLSSVIIGAAWPLMLERFSVQPNRAEKEAEYISRNIESTRYAYGITDEDVTYEENWGAGETTNEEVAADSATISNIRLLDPQILSPTFTQQQQLRNFYGFPDQLAMDRFEVDGKLRDFVVAARELDPNALQQNQQDWINRHTVYTHGNGFIAAQANQVDEVARDVGSTRGGYPVYTVSDLQSNARAAESEDAEELGIKVDEPRVYYGPLIASATDGADYAIVGDTGDGPVEYDTDTSSYTYEGAGGVDIGNMVNRAMFALRYQEMNMLLSDRVGSESKILFERDPRSRVEKVAPWLTTDSKTYPTVIDGRIKWIVDGYTTLDSLPYSTRTSLTEATQDAVMPDGTPQPLITDRVGYIRNSVKAVVDAYDGTVELYEFDTEDPVLKAWRGVFPDTVKDGSEISDELRAHLRYPEDLFKVQRDMLAKYNVDDSGTFFTNDAFWSVPGDPTAAEGRQELKQPPYYVVAADPETGESSFQLITPFRGLQREYLSAHMSASSDPVTYGEITVRVLPTDSVTQGPKQAQDAMMSSDQVAQDQTLWRGSNDLHNGNLLTLPVGGGEILYVEPIYSQRKDQASAFPKLLRVLVFYKGQVGYAPTIAEALSQVGIDPKEAQDIEEVDGTATTPSTDETDTDTDQPATETPTAPVSEAEGIAAINDALSNLEAARDSSFEEYGRALDALDRAVDSYQSAQ

SEQ ID NO: 4 - DNA, 2958 bp, Artificial Sequence
  (WT)_NCgl0752_nucleic acid
ttgtcgactggtctcacacctcctccccaaccgatcaagcgacctcccaaggcggtgacatggatcttcgccattatcgcgttggtcattctcatcgccccaatgagtgttggcttctataccgactggctttggttcggtgaagtcgatttccgaggcgttttcagcaaggttattgtcactcgcattgttctctttgtgatctttgcgctaattgctgggtttgtcacatggcttgctggttattttgtgacaaaacttcgacctgatgagatgtcggcgtttgatacccagtcgcctgtgtatcagtaccgtcagatgatcgaaaacagccttcgtcgcgttatggtgatcattccaattttcgtcgcgttgctggctggcctaattggtcagcgttcgtggcgcaccgttcaaatgtggctgaatggccaggactttggcgtttcggatcagcagttcggcttggattatggattctacgcgtttgatcttccgatgcttcgcctcatcgctgactcactgtcgatgatgttgatcgttgctttcctgatcgcactcgttggccattacctcatgggtggcattcgcgctggaaaccagatgacgggccagaagtcctttgtatcccgtggtgcgcgcactcagcttgcggtaactgctggtctgtggatgcttgttaaggtcgctggctactggctggatcgctatgacctgctgactaaggaaaactcaaccttcacaggtgcaagctacaccgacatcaatgcacagctgccagcgaagatcatcctgctggttatcgcattgttcgtggcgatcgcgttcttctctgcgatcttcctgaaggacctccgcatcccaggtcttgccgtagttctgatgctgctgagctctgtgatcattggtgctgcttggcctttgatgctggagcgtttctccgttcagccaaaccgtgcagaaaaagaagccgagtacatttctcgaaacattgaatcgactcgctatgcctatggcatcaccgatgaagatgtcacctacgaggaaaactggggagcaggggagaccaccaatgaagaagtcgccgctgattctgcaacgatttctaacattcgtctgctggatccacagatcctgtcaccaaccttcacccagcaacagcagctgcgaaacttctacggtttcccagaccagctggcgatggaccgctttgaagtagatggcaaactccgcgactttgttgtggcagcacgtgagctcgatccaaacgccctgcagcaaaaccagcaggactggattaaccgtcacactgtttatacccacggcaacggcttcattgcagctcaagcaaaccaggtggatgaggtcgcccgcgacgtcggatccactcgtggtggttaccctgtctacaccgtctctgatttgcagtcgaatgctcgtgctgcagaaagcgaagatgctgaggagcttggcatcaaggttgatgagcctcgtgtgtactacggaccactgattgcttctgcgactgatggtgctgactacgcaattgtcggtgacaccggcgatggcccagtcgagtacgacactgacacctccagctacacctacgaaggtgctggcggcgtggacattggaaacatggtcaaccgtgcgatgtttgcattgcgctaccaggaaatgaacatgctcctgtctgatcgtgttggttccgaatccaagatcctatttgagcgcgatcctcgttcccgtgtggaaaaggttgcaccttggttgaccactgactccaagacctacccaactgtgattgatggtcgcatcaagtggatcgtcgatggctacaccaccttggatagtcttccgtactccacgcgcacctcactgacggaagcgactcaggatgctgtcatgcctgacggcaccccacagccactgatcacagatagggtcggttacatccgcaactccgtgaaggctgttgttgatgcgtacgacggaactgttgaactctacgaattcgacaccgaagatcctgttctgaaggcatggcgtggcgtgttcccagacaccgtgaaggacgggtcggagatttccgatgagcttcgcgcacacctgcgttacccagaagatttgttcaaggtccagcgtgacatgctggccaagtacaacgttgatgattctggaacattcttcaccaacgatgcgttctggtctgtcccaggtgacccaactgcagcggagggccgccaggaacttaagcagcctccttactacgtggtggcagcagacccagagaccggtgagtccagcttccagctgatcaccccgttccgtggacttcagcgcgagtacctctctgcacacatgtctgcgtcgtctgatccagttacctacggtgaaatcactgttcgtgtgctgcctaccgattctgtgacccagggtccaaagcaggcccaggatgcgatgatgtcatctgaccaggttgctcaggaccaaacactgtggcgtggatcgaacgatctgcacaacggaaacctgttgaccttgccagttggtggcggagagatcctctacgttgagccgatttactcgcagcgcaaggatcaggcatcggccttcccgaagcttctgcgcgtgctggtcttctacaagggtcaggttggttacgcaccaacgatcgctgaagccctatcgcaggtcggcattgatccgaaggaagcgcaggacatcgaagaggtagatggcaccgctacgacgccatcgactgatgagactgacactgacactgatcagcctgcaaccgaaaccccaactgcaccagtgagtgaggcggaaggaatcgcggccatcaacgatgcgttgagcaaccttgaagctgctcgcgatagctctttcgaagagtatggtcgtgcactcgatgcgcttgatcgtgccgtcgatagctaccagtccgcacagtag

SEQ ID NO: 5 - DNA, 38 bp, Artificial Sequence
  NCgl0752_1F
tgaattcgagctcggtacccgctgaggagcttggcatc

SEQ ID NO: 6 - DNA, 33 bp, Artificial Sequence
  NCgl0752_2R
gccttcagaacaggatattcggtgtcgaattcg

SEQ ID NO: 7 - DNA, 33 bp, Artificial Sequence
  NCgl0752_3F
cgaattcgacaccgaatatcctgttctgaaggc

SEQ ID NO: 8 - DNA, 36 bp, Artificial Sequence
  NCgl0752_4R
gtcgactctagaggatcccccgatcctctcgggctg

SEQ ID NO: 9 - DNA, 17 bp, Artificial Sequence
  NCgl0752_5F
ggatccactcgtggtgg

SEQ ID NO: 10 - DNA, 18 bp, Artificial Sequence
  NCgl0752_6R
gatgcggtgtctctaggc